European Patent Application EP 4 556 018 A1, published May 21, 2025. Title: 腫瘍の予防および／または治療剤. Applicant: 国立大学法人大阪大学. The sequence listing filed with the application follows.

SEQUENCE LISTING (18 sequences)

SEQ ID NO: 1 - protein, 535 aa, Mus musculus
MDVDEGQDMSQVSGKESPPVSDTPDEGDEPMPVPEDLSTTSGAQQNSKSDRGMVAYGADGFRDFHAIIPKSFSPSNVKVETQSDEENGRACEMNGEECAEDLRMLDASGEKMNGSHRDQGSSALSGVGGIRLPNGKLKCDICGIVCIGPNVLMVHKRSHTGERPFQCNQCGASFTQKGNLLRHIKLHSGEKPFKCHLCNYACRRRDALTGHLRTHSVGKPHKCGYCGRSYKQRSSLEEHKERCHNYLESMGLPGMYPVIKEETNHNEMAEDLCKIGAERSLVLDRLASNVAKRKSSMPQKFLGDKCLSDMPYDSANYEKEDMMTSHVMDQAINNAINYLGAESLRPLVQTPPGSSEVVPVISSMYQLHKPPSDGPPRSNHSAQDAVDNLLLLSKAKSVSSEREASPSNSCQDSTDTESNAEEQRSGLIYLTNHINPHARNGLALKEEQRAYEVLRAASENSQDAFRVVSTSGEQLKVYKCEHCRVLFLDHVMYTIHMGCHGFRDPFECNMCGYHSQDRYEFSSHITRGEHRYHLS

SEQ ID NO: 2 - protein, 429 aa, Mus musculus
MPNPRPAKPMAPSLALGPSPGVLPSWKTAPKGSELLGTRGSGGPFQGRDLRSGAHTSSSLNPLPPSQLQLPTVPLVMVAPSGARLGPSPHLQALLQDRPHFMHQLSTVDAHAQTPVLQVRPLDNPAMISLPPPSAATGVFSLKARPGLPPGINVASLEWVSREPALLCTFPRSGTPRKDSNLLAAPQGSYPLLANGVCKWPGCEKVFEEPEEFLKHCQADHLLDEKGKAQCLLQREVVQSLEQQLELEKEKLGAMQAHLAGKMALAKAPSVASMDKSSCCIVATSTQGSVLPAWSAPREAPDGGLFAVRRHLWGSHGNSSFPEFFHNMDYFKYHNMRPPFTYATLIRWAILEAPERQRTLNEIYHWFTRMFAYFRNHPATWKNAIRHNLSLHKCFVRVESEKGAVWTVDEFEFRKKRSQRPNKCSNPCP

SEQ ID NO: 3 - protein, 539 aa, Homo sapience
MDADEGQDMSQVSGKESPPVSDTPDEGDEPMPIPEDLSTTSGGQQSSKSDRVVVTYGADDFRDFHAIIPKSFSPSNVKVETQSDEENGRACEMNGEECAEDLRMLDASGEKMNGSHRDQGSSALSGVGGIRLPNGKLKCDICGIICIGPNVLMVHKRSHTGERPFQCNQCGASFTQKGNLLRHIKLHSGEKPFKCHLCNYACRRRDALTGHLRTHSVGKPHKCGYCGRSYKQRSSLEEHKERCHNYLESMGLPGTLYPVIKEETNHSEMAEDLCKIGSERSLVLDRLASNVAKRKSSMPQKFLGDKGLSDTPYDSSASYEKENEMMKSHVMDQAINNAINYLGAESLRPLVQTPPGGSEVVPVISPMYQLHKPLAEGTPRSNHSAQDSAVENLLLLSKAKLVPSEREASPSNSCQDSTDTESNNEEQRSGLIYLTNHIAPHARNGLSLKEEHRAYDLLRAASENSQDALRVVSTSGEQMKVYKCEHCRVLFLDHVMYTIHMGCHGFRDPFECNMCGYHSQDRYEFSSHITRGEHRFHMS

SEQ ID NO: 4 - protein, 431 aa, Homo sapience
MPNPRPGKPSAPSLALGPSPGASPSWRAAPKASDLLGARGPGGTFQGRDLRGGAHASSSSLNPMPPSQLQLPTLPLVMVAPSGARLGPLPHLQALLQDRPHFMHQLSTVDAHARTPVLQVHPLESPAMISLTPPTTATGVFSLKARPGLPPGINVASLEWVSREPALLCTFPNPSAPRKDSTLSAVPQSSYPLLANGVCKWPGCEKVFEEPEDFLKHCQADHLLDEKGRAQCLLQREMVQSLEQQLVLEKEKLSAMQAHLAGKMALTKASSVASSDKGSCCIVAAGSQGPVVPAWSGPREAPDSLFAVRRHLWGSHGNSTFPEFLHNMDYFKFHNMRPPFTYATLIRWAILEAPEKQRTLNEIYHWFTRMFAFFRNHPATWKNAIRHNLSLHKCFVRVESEKGAVWTVDELEFRKKRSQRPSRCSNPTPGP

SEQ ID NO: 5 - RNA, 23 nt, synthetic construct
  source 1..23: mol_type = other RNA
agagcgatgccacaactacttgg

SEQ ID NO: 6 - RNA, 23 nt, synthetic construct
  source 1..23: mol_type = other RNA
cagaactccaagagtgatcgagg

SEQ ID NO: 7 - RNA, 23 nt, synthetic construct
  source 1..23: mol_type = other RNA
agatgaactgcgacgtgtgcggg

SEQ ID NO: 8 - RNA, 23 nt, synthetic construct
  source 1..23: mol_type = other RNA
attatgaagccggagcccatggg

SEQ ID NO: 9 - RNA, 23 nt, synthetic construct
  source 1..23: mol_type = other RNA
cgactatgaaagcattaagctgg

SEQ ID NO: 10 - protein, 56 aa, Homo sapience
GERPFQCNQCGASFTQKGNLLRHIKLHSGEKPFKCHLCNYACRRRDALTGHLRTHS

SEQ ID NO: 11 - RNA, 23 nt, synthetic construct
  source 1..23: mol_type = other RNA
cgaaggggaacacgccaatatgg

SEQ ID NO: 12 - RNA, 23 nt, synthetic construct
  source 1..23: mol_type = other RNA
gggtaaaagaagctccgcactgg

SEQ ID NO: 13 - RNA, 23 nt, synthetic construct
  source 1..23: mol_type = other RNA
tcagtttaccattcggaagccgg

SEQ ID NO: 14 - RNA, 23 nt, synthetic construct
  source 1..23: mol_type = other RNA
aagctcaagtgcgacgtctgcgg

SEQ ID NO: 15 - RNA, 23 nt, synthetic construct
  source 1..23: mol_type = other RNA
cttgtagggtttgcccacggtgg

SEQ ID NO: 16 - RNA, 23 nt, synthetic construct
  source 1..23: mol_type = other RNA
ttatccaggagccgttcatccgg

SEQ ID NO: 17 - protein, 23 aa, Homo sapiens
QCNQCGASFTQKGNLLRHIKLHS

SEQ ID NO: 18 - protein, 23 aa, Homo sapiens
KCHLCNYACRRRDALTGHLRTHS